European Patent Application EP 4 538 287 A1, published April 16, 2025. Title: Novel Engineered Anti-Streptococcus Antibodies. Applicant: Tanea Medical AB. Application EP, filed October 6, 2023. The sequence listing filed with the application follows.

SEQUENCE LISTING (15 sequences)

SEQ ID NO: 1 - protein, 377 aa, Homo sapiens
ASTKGPSVFPLAPCSRSTSGGTAALGCLVKDYFPEPVTVSWNSGALTSGVHTFPAVLQSSGLYSLSSVVTVPSSSLGTQTYTCNVNHKPSNTKVDKRVELKTPLGDTTHTCPRCPEPKSCDTPPPCPRCPEPKSCDTPPPCPRCPEPKSCDTPPPCPRCPAPELLGGPSVFLFPPKPKDTLMISRTPEVTCVVVDVSHEDPEVQFKWYVDGVEVHNAKTKPREEQFNSTFRVVSVLTVLHQDWLNGKEYKCKVSNKALPAPIEKTISKTKGQPREPQVYTLPPSREEMTKNQVSLTCLVKGFYPSDIAVEWESSGQPENNYNTTPPMLDSDGSFFLYSKLTVDKSRWQQGNIFSCSVMHEALHNRFTQKSLSLSPGK

SEQ ID NO: 2 - protein, 377 aa, Synthetic construct
ASTKGPSVFPLAPCSRSTSGGTAALGCLVKDYFPEPVTVSWNSGALTSGVHTFPAVLQSSGLYSLSSVVTVPSSSLGTQTYTCNVNHKPSNTKVDKRVELKTPLGDTTHTCPRCPEPKSCDTPPPCPRCPEPKSCDTPPPCPRCPEPKSCDTPPPCPRCPAPELLGGPSVFLFPPKPKDTLMISRTPEVTCVVVDVSHEDPEVQFKWYVDGVEVHNAKTKPREEQFNSTFRVVSVLTVLHQDWLNGKEYKCKVSNKALPAPIEKTISKTKGQPREPQVYTLPPSREEMTKNQVSLTCLVKGFYPSDIAVEWESSGQPENNYKTTPPVLDSDGSFFLYSKLTVDKSRWQQGNIFSCSVMHEALHNHFTQKSLSLSPGK

SEQ ID NO: 3 - protein, 362 aa, Synthetic construct
ASTKGPSVFPLAPSSKSTSGGTAALGCLVKDYFPEPVTVSWNSGALTSGVHTFPAVLQSSGLYSLSSVVTVPSSSLGTQTYICNVNHKPSNTKVDKKVELKTPLGDTTHTCPRCPEPKSCDTPPPCPRCPEPKSCDTPPPCPRCPAPELLGGPSVFLFPPKPKDTLMISRTPEVTCVVVDVSHEDPEVKFNWYVDGVEVHNAKTKPREEQYNSTYRVVSVLTVLHQDWLNGKEYKCKVSNKALPAPIEKTISKAKGQPREPQVYTLPPSRDELTKNQVSLTCLVKGFYPSDIAVEWESNGQPENNYKTTPPVLDSDGSFFLYSKLTVDKSRWQQGNVFSCSVMHEALHNHYTQKSLSLSPGK

SEQ ID NO: 4 - protein, 62 aa, Synthetic construct
ELKTPLGDTTHTCPRCPEPKSCDTPPPCPRCPEPKSCDTPPPCPRCPEPKSCDTPPPCPRCP

SEQ ID NO: 5 - protein, 17 aa, Synthetic construct
ELKTPLGDTTHTCPRCP

SEQ ID NO: 6 - protein, 15 aa, Synthetic construct
EPSKCDTPPPCPRCP

SEQ ID NO: 7 - protein, 18 aa, Homo sapiens
CARSYPHKRWLRPPFDYW

SEQ ID NO: 8 - protein, 18 aa, Homo sapiens
CAKNSRSGWYFFFDYWGQ

SEQ ID NO: 9 - protein, 18 aa, Homo sapiens
CARQGFDTRGEDAFEIWG

SEQ ID NO: 10 - protein, 18 aa, Homo sapiens
CVRDSRFWGIFDYWGQGT

SEQ ID NO: 11 - protein, 15 aa, Homo sapiens
QYNSYPVTFGQGTKV

SEQ ID NO: 12 - protein, 15 aa, Homo sapiens
QYDNLPLTFGGGTKV

SEQ ID NO: 13 - protein, 17 aa, Homo sapiens
QRSGWPSIFTFGPGTKV

SEQ ID NO: 14 - protein, 15 aa, Homo sapiens
QRSNWPPTFGQGTKV

SEQ ID NO: 15 - protein, 47 aa, Synthetic construct
ELKTPLGDTTHTCPRCPEPSKCDTPPPCPRCPEPSKCDTPPPCPRCP